European Patent Application EP 4 123 017 A1, published January 25, 2023. Title: Composition comprising a cardiac stem cell for the prevention and treatment of ischemic disease. Applicant: HieraBio Inc. The sequence listing filed with the application follows.

SEQUENCE LISTING (12 sequences)

SEQ ID NO: 1 - DNA, 23 bp, Artificial Sequence
  VEGF forward primer
ggagtaccccgatgagatagagt

SEQ ID NO: 2 - DNA, 21 bp, Artificial Sequence
  VEGF reverse primer
ctatgtgctggctttggtgag

SEQ ID NO: 3 - DNA, 20 bp, Artificial Sequence
  PDGF-B forward primer
tggagtcgagtcggaaagct

SEQ ID NO: 4 - DNA, 20 bp, Artificial Sequence
  PDGF-B reverse primer
gaagttggcattggtgcgat

SEQ ID NO: 5 - DNA, 20 bp, Artificial Sequence
  bFGF forward primer
gcgacccacacgtcaaacta

SEQ ID NO: 6 - DNA, 20 bp, Artificial Sequence
  bFGF reverse primer
cagccgtccatcttccttca

SEQ ID NO: 7 - DNA, 22 bp, Artificial Sequence
  Ang-1 forward primer
ctcgctgccattctgactacac

SEQ ID NO: 8 - DNA, 21 bp, Artificial Sequence
  Ang-1 reverse primer
gacagttgccatcgtgttctg

SEQ ID NO: 9 - DNA, 23 bp, Artificial Sequence
  beta-actin forward primer
agatcaagatcattgctcctcct

SEQ ID NO: 10 - DNA, 20 bp, Artificial Sequence
  beta-actin reverse primer
acgcagctcagtaacagtcc

SEQ ID NO: 11 - protein, 823 aa, Artificial Sequence
  HIF-1 protein
MEGAGGENEKKNRMSSERRKEKSRDAARSRRSKESEVFYELAHQLPLPHNVSSHLDKASVMRLTISYLRVRKLLGAGDLDIEDEMKAQMNCFYLKALDGFVMVLTDDGDMIYISDNVNKYMGLTQFELTGHSVFDFTHPCDHEEMREMLTHRNGPVRKGKEQNTQRSFFLRMKCTLTSRGRTMNIKSATWKVLHCTGHIHVYDTSSNQPQCGYKKPPMTCLVLICEPIPHPSNIEIPLDSKTFLSRHSLDMKFSYCDERITELMGYEPEELLGRSIYEYYHALDSDHLTKTHHDMFTKGQVTTGQYRMLAKRGGYVWVETQATVIYNTKNSQPQCIVCVNYVVSGIIQHDLIFSLQQTESVLKPVESSDMKMTQLFTKVESEDTSCLFDKLKKEPDALTLLAPAAGDTIISLDFGSDDTETEDQQLEDVPLYNDVMFPSSNEKLNINLAMSPLPASETPKPLRSSADPALNQEVALKLESSPESLGLSFTMPQIQDQPASPSDGSTRQSSPEPNSPSEYCFDVDSDMVNVFKLELVEKLFAEDTEAKNPFSAQDTDLDLEMLAPYIPMDDDFQLRSFDQLSPLESNSPSPPSVSTVTGFQQTQLQKPTITVTATATATTDESKAVTKDNIEDIKILIASPPSTQVPQEMTTAKASAYSGTHSRTASPDRAGKRVIEKTDKAHPRSLNLSVTLNQRNTVPEEELNPKTIALQNAQRKRKMEHDGSLFQAAGIGTLLQQPGDRAPTMSLSWKRVKGYISSEQDGMEQKTIFLIPSDLACRLLGQSMDESGLPQLTSYDCEVNAPIQGSRNLLQGEELLRALDQVN

SEQ ID NO: 12 - protein, 696 aa, Artificial Sequence
  constitutively active HIF-1 protein
MEGAGGANDKKKISSERRKEKSRDAARSRRSKESEVFYELAHQLPLPHNVSSHLDKASVMRLTISYLRVRKLLDAGDLDIEDDMKAQMNCFYLKALDGFVMVLTDDGDMIYISDNVNKYMGLTQFELTGHSVFDFTHPCDHEEMREMLTHRNGLVKKGKEQNTQRSFFLRMKCTLTSRGRTMNIKSATWKVLHCTGHIHVYDTNSNQPQCGYKKPPMTCLVLICEPIPHPSNIEIPLDSKTFLSRHSLDMKFSYCDERITELMGYEPEELLGRSIYEYYHALDSDHLTKTHHDMFTKGQVTTGQYRMLAKRGGYVWVETQATVIYNTKNSQPQCIVCVNYVVSGIIQHDLIFSLQQTECVLKPVESSDMKMTQLFTKVESEDTSSLFDKLKFYVDSDMVNEFKLELVEKLFAEDTEAKNPFSTQDTDLDLEMLAPYITDDDFQLRSFDQLSPLESSSASPESASPQSTVTVFQQTQIQEPTANATTTTATTDELKTVTKDRMEDIKILIASPSPTHIHKETTSATSSQYRDTQSRTASPNRAGKGVIEQTEKSHPRSPNVLSVALSQRTTVPEEELNPKILALQNAQRKRKMEHDGSLFQAVGIGTLLQQPDDHAATTSLSWKRVKGCKSSEQNGMEQKTIILIPSDLACRLLGQSMDESGLPQLTSYDCEVNAPIQGSRNLLQGEELLRALDQVN